European Patent Application EP 4 166 648 A1, published April 19, 2023. Title: A YEAST AND LACTIC ACID BACTERIA COMBINATION. Applicant: Mingzhiyuan (Hangzhou) Biological Technology Co., Ltd. Application CN 202111198135.X, filed October 14, 2021. The sequence listing filed with the application follows.

SEQUENCE LISTING (6 sequences)

SEQ ID NO: 1 - DNA, 1654 bp, Artificial Sequence
  source 1..1654: mol_type = other DNA
agtatagcattatacggtgaaactgcgaatggctcattaaatcagttatcgtttatttgatagttccgttctacatggataaccgtggaaaatctagagctaatacatgcgtaaagccccgacttttggaggggtgtatttattagataaaaaatcaatgccctcgggccttttgatgattcataataacttttcgaagcccatggccttgtgccggcggctggttcattcaaatttctgccctatcaactttcgatggtaggatagaggcctaccatggttttcacgggtaacggggaataagggttcgattccggagagggagcctgagaaacggctaccacatccaaggaaggcagcaggcgcgcaaattacccaatcctgacacagggaggtagtgacaatatataacgatacagggccattggtcttgtaattggaatgagtacaatgtaaataccttaacgaggaacaattggagggcaagtctggtgccagcagccgcggtaattccagctccaatagcgtatattaaagttgttgcagttaaaaagctcgtagttgaagtttgggcctgggcgggcggtctacctatggtgagtactgcagcggccgggtctttccttctggctagccctcgtggcgaaccaggacgattactttgaggaaattagagtgttcaaagcaggcctttgctcggatatattagcatggaataatagaataggacgtatggttctattttgttggtttctaggaccatcgtaatgattaatagggacggtcgggggcatcagtattcagttgtcagaggtgaaattcttggattaactgaagactaactactgcgaaagcatttgccaaggacgttttcattaatcaagaacgaaagttaggggatcgaagatgatcagataccgtcgtagtcttaaccataaactatgccgactagggatcgggtggcgctttgtggcccatccggcaccttgtgagaaatcaaagtctttgggttctggggggagtatggttgcaaggctgaaacttaaaggaattgacggaagggcaccaccaggagtggagcctgcggcttaatttgactcaacacggggaaactcaccaggtccagacgtaataaggattgacaagttagagacttctcttgatcttacgggtggtggtgcatggccgtttttagtccttggagtgatttgtctgcttaattgcgataacggacgagaccttaacctgctaaatagggctgcgagcatctgcttgtgggctcttcttagagggactatgggtatcaaacccatggaagtttgaggcaacaacaggtctgtgatgcccttagacgttctgggccgcacgcgcgctacactgacggagccagcaagtacaaccttggtcgagaggcccgggtaatctcgtgaaactccgtcgtgctggggatagagcattgtaatttttgctcttcaacgaggaattcctagtaagcgcaagtcatcagcttgcgttgattacgtccctgccctttgtacacaccgcccgtcgctactaccgattgaatggcttagtgaggcttcaggattggcgccgcgggaggggcaactttgccatggcgccgagaatctagacaaacttggtcattagaggt

SEQ ID NO: 2 - DNA, 1457 bp, Artificial Sequence
  source 1..1457: mol_type = other DNA
tgcaagtcgaacgcgtctccgttaatgattttaggtgcttgcacttgaaagatttaacattgagacgagtggcgaactggtgagtaacacgtgggtaacctgcccttgaagtaggggataacacttggaaacaggtgctaataccgtataacaaccaaaaccacctggttttggtttaaaagacggcttcggctgtcactttaggatggacccgcggcgtattagcttgttggtaaggtaacggcttaccaaggcgatgatacgtagccgacctgagagggtaatcggccacattgggactgagacacggcccaaactcctacgggaggcagcagtagggaatcttccacaatggacgaaagtctgatggagcaacgccgcgtgagtgatgaagggtttcggctcgtaaaactctgttgttggagaagaacaggtgtcagagtaactgttgacatcttgacggtatccaaccagaaagccacggctaactacgtgccagcagccgcggtaatacgtaggtggcaagcgttgtccggatttattgggcgtaaagcgagcgcaggcggttttttaggtctgatgtgaaagccttcggcttaaccggagaagtgcatcggaaaccgggagacttgagtgcagaagaggacagtggaactccatgtgtagcggtgaaatgcgtagatatatggaagaacaccagtggcgaaggcggctgtctggtctgtaactgacgctgaggctcgaaagcatgggtagcgaacaggattagataccctggtagtccatgccgtaaacgatgagtgctaagtgttggagggtttccgcccttcagtgctgcagctaacgcattaagcactccgcctggggagtacgaccgcaaggttgaaactcaaaggaattgacgggggcccgcacaagcggtggagcatgtggtttaattcgatgctacgcgaagaaccttaccaggtcttgacatcttctgccaacttaagagattaggcgttcccttcggggacagaatgacaggtggtgcatggttgtcgtcagctcgtgtcgtgagatgttgggttaagtcccgcaacgagcgcaacccttattgttagttgccagcattcagttgggcactctagcaagactgccggtgacaaaccggaggaaggtggggatgacgtcaaatcatcatgccccttatgacctgggctacacacgtgctacaatggacggtacaacgagtcgcgaaaccgcgaggtcaagctaatctcttaaagccgttctcagttcggattgtaggctgcaactcgcctacatgaagttggaatcgctagtaatcgtggatcagcatgccacggtgaatacgttcccgggccttgtacacaccgcccgtcacaccatgagagtttgtaacacccaaagccggtgaggtaaccttcggggaccagccgtctaaggtgacagga

SEQ ID NO: 3 - DNA, 1454 bp, Artificial Sequence
  source 1..1454: mol_type = other DNA
gcgtgctatactgcaagtcgaacgagttctcgttgatgatcggtgcttgcaccgagattcaacatggaacgagtggcggacgggtgagtaacacgtgggtaacctgcccttaagtgggggataacatttggaaacagatgctaataccgcatagatccaagaaccgcatggttcttggctgaaagatggcgtaagctatcgcttttggatggacccgcggcgtattagctagttggtgaggtaatggctcaccaaggcgatgatacgtagccgaactgagaggttgatcggccacattgggactgagacacggcccaaactcctacgggaggcagcagtagggaatcttccacaatggacgcaagtctgatggagcaacgccgcgtgagtgaagaaggctttcgggtcgtaaaactctgttgttggagaagaatggtcggcagagtaactgttgtcggcgtgacggtatccaaccagaaagccacggctaactacgtgccagcagccgcggtaatacgtaggtggcaagcgttatccggatttattgggcgtaaagcgagcgcaggcggttttttaagtctgatgtgaaagccctcggcttaaccgaggaagcgcatcggaaactgggaaacttgagtgcagaagaggacagtggaactccatgtgtagcggtgaaatgcgtagatatatggaagaacaccagtggcgaaggcggctgtctggtctgtaactgacgctgaggctcgaaagcatgggtagcgaacaggattagataccctggtagtccatgccgtaaacgatgaatgctaggtgttggagggtttccgcccttcagtgccgcagctaacgcattaagcattccgcctggggagtacgaccgcaaggttgaaactcaaaggaattgacgggggcccgcacaagcggtggagcatgtggtttaattcgaagcaacgcgaagaaccttaccaggtcttgacatcttttgatcacctgagagatcaggtttccccttcgggggcaaaatgacaggtggtgcatggttgtcgtcagctcgtgtcgtgagatgttgggttaagtcccgcaacgagcgcaacccttatgactagttgccagcatttagttgggcactctagtaagactgccggtgacaaaccggaggaaggtggggatgacgtcaaatcatcatgccccttatgacctgggctacacacgtgctacaatggatggtacaacgagttgcgagaccgcgaggtcaagctaatctcttaaagccattctcagttcggactgtaggctgcaactcgcctacacgaagtcggaatcgctagtaatcgcggatcagcacgccgcggtgaatacgttcccgggccttgtacacaccgcccgtcacaccatgagagtttgtaacacccgaagccggtggcgtaacccttttagggagcgagccgtctaag

SEQ ID NO: 4 - DNA, 1460 bp, Artificial Sequence
  source 1..1460: mol_type = other DNA
cgccttgcgtgctatacatgcagtcgaacgagttttggtcgatgaacggtgcttgcattgtgattcaacttaaaacgagtggcggacgggtgagtaacacgtgggtaacctgcccttaagtgggggataacatttggaaacagatgctaataccgcataaatccaagaaccgcatggttcttggctgaaagatggcgcaagctatcgcttttggatggacccgcggcgtattagctagttggtgaggtaacggctcaccaaggcgatgatacgtagccgaactgagaggttgatcggccacattgggactgagacacggcccaaactcctacgggaggcagcagtagggaatcttccacaatggacgcaagtctgatggagcaacgccgcgtgagtgaagaaggctttcgggtcgtaaaactctgttgttggagaagaatggtcggcagagtaactgttgtcggcgtgacggtatccaaccagaaagccacggctaactacgtgccagcagccgcggtaatacgtaggtggcaagcgttatccggatttattgggcgtaaagcgagcgcaggcggttttttaagtctgatgtgaaagccctcggcttaaccgaggaagcgcatcggaaactgggaaacttgagtgcagaagaggacagtggaactccatgtgtagcggtgaaatgcgtagatatatggaagaacaccagtggcgaaggcggctgtctggtctgtaactgacgctgaggctcgaaagcatgggtagcgaacaggattagataccctggtagtccatgccgtaaacgatgaatgctaggtgttggagggtttccgcccttcagtgccgcagctaacgcattaagcattccgcctggggagtacgaccgcaaggttgaaactcaaaggaattgacgggggcccgcacaagcggtggagcatgtggtttaattcgaagcaacgcgaagaaccttaccaggtcttgacatcttttgatcacctgagagatcaggtttccccttcgggggcaaaatgacaggtggtgcatggttgtcgtcagctcgtgtcgtgagatgttgggttaagtcccgcaacgagcgcaacccttatgactagttgccagcattcagttgggcactctagtaagactgccggtgacaaaccggaggaaggtggggatgacgtcaaatcatcatgccccttatgacctgggctacacacgtgctacaatggatggtacaacgagttgcgagaccgcgaggtcaagctaatctcttaaagccattctcagttcggactgtaggctgcaactcgcctacacgaagtcggaatcgctagtaatcgcggatcagcacgccgcggtgaatacgttcccgggccttgtacacaccgcccgtcacaccatgagagtttgtaacacccgaagccggtggcgtaacccttttagggagcgagccgtctaag

SEQ ID NO: 5 - DNA, 1452 bp, Artificial Sequence
  source 1..1452: mol_type = other DNA
tgggtgctatacatgcagtcgaacgaactctggtattgattggtgcttgcatcatgatttacatttgagtgagtggcgaactggtgagtaacacgtgggaaacctgcccagaagcgggggataacacctggaaacagatgctaataccgcataacaacttggaccgcatggtccgagcttgaaagatggcttcggctatcacttttggatggtcccgcggcgtattagctagatggtggggtaacggctcaccatggcaatgatacgtagccgacctgagagggtaatcggccacattgggactgagacacggcccaaactcctacgggaggcagcagtagggaatcttccacaatggacgaaagtctgatggagcaacgccgcgtgagtgaagaagggtttcggctcgtaaaactctgttgttaaagaagaacatatctgagagtaactgttcaggtattgacggtatttaaccagaaagccacggctaactacgtgccagcagccgcggtaatacgtaggtggcaagcgttgtccggatttattgggcgtaaagcgagcgcaggcggttttttaagtctgatgtgaaagccttcggctcaaccgaagaagtgcatcggaaactgggaaacttgagtgcagaagaggacagtggaactccatgtgtagcggtgaaatgcgtagatatatggaagaacaccagtggcgaaggcggctgtctggtctgtaactgacgctgaggctcgaaagtatgggtagcaaacaggattagataccctggtagtccataccgtaaacgatgaatgctaagtgttggagggtttccgcccttcagtgctgcagctaacgcattaagcattccgcctggggagtacggccgcaaggctgaaactcaaaggaattgacgggggcccgcacaagcggtggagcatgtggtttaattcgaagctacgcgaagaaccttaccaggtcttgacatactatgcaaatctaagagattagacgttcccttcggggacatggatacaggtggtgcatggttgtcgtcagctcgtgtcgtgagatgttgggttaagtcccgcaacgagcgcaacccttattatcagttgccagcattaagttgggcactctggtgagactgccggtgacaaaccggaggaaggtggggatgacgtcaaatcatcatgccccttatgacctgggctacacacgtgctacaatggatggtacaacgagttgcgaactcgcgagagtaagctaatctcttaaagccattctcagttcggattgtaggctgcaactcgcctacatgaagtcggaatcgctagtaatcgcggatcagcatgccgcggtgaatacgttcccgggccttgtacacaccgcccgtcacaccatgagagtttgtaacacccaaagtcggtggggtaaccttttaggaaccagccgcctaag

SEQ ID NO: 6 - DNA, 1456 bp, Artificial Sequence
  source 1..1456: mol_type = other DNA
gcgtgctatactgcagtcgaacgagttttggtcgatgaacggtgcttgcactgtgattcaacttaaaacgagtggcggacgggtgagtaacacgtgggtaacctgcccttaagtgggggataacatttggaaacagatgctaataccgcataaatccaagaaccgcatggttcttggctgaaagatggcgtaagctatcgcttttggatggacccgcggcgtattagctagttggtgaggtaacggctcaccaaggcgatgatacgtagccgaactgagaggttgatcggccacattgggactgagacacggcccaaactcctacgggaggcagcagtagggaatcttccacaatggacgcaagtctgatggagcaacgccgcgtgagtgaagaaggctttcgggtcgtaaaactctgttgttggagaagaatggtcggcagagtaactgttgtcggcgtgacggtatccaaccagaaagccacggctaactacgtgccagcagccgcggtaatacgtaggtggcaagcgttatccggatttattgggcgtaaagcgagcgcaggcggttttttaagtctgatgtgaaagccctcggcttaaccgaggaagcgcatcggaaactgggaaacttgagtgcagaagaggacagtggaactccatgtgtagcggtgaaatgcgtagatatatggaagaacaccagtggcgaaggcggctgtctggtctgtaactgacgctgaggctcgaaagcatgggtagcgaacaggattagataccctggtagtccatgccgtaaacgatgaatgctaggtgttggagggtttccgcccttcagtgccgcagctaacgcattaagcattccgcctggggagtacgaccgcaaggttgaaactcaaaggaattgacgggggcccgcacaagcggtggagcatgtggtttaattcgaagcaacgcgaagaaccttaccaggtcttgacatcttttgatcacctgagagatcaggtttccccttcgggggcaaaatgacaggtggtgcatggttgtcgtcagctcgtgtcgtgagatgttgggttaagtcccgcaacgagcgcaacccttatgactagttgccagcattcagttgggcactctagtaagactgccggtgacaaaccggaggaaggtggggatgacgtcaaatcatcatgccccttatgacctgggctacacacgtgctacaatggatggtacaacgagttgcgagaccgcgaggtcaagctaatctcttaaagccattctcagttcggactgtaggctgcaactcgcctacacgaagtcggaatcgctagtaatcgcggatcagcacgccgcggtgaatacgttcccgggccttgtacacaccgcccgtcacaccatgagagtttgtaacacccgaagccggtggcgtaacccttttaggagcgagccgtcaagtgaca